European Patent Application EP 4 513 189 A1, published February 26, 2025. Title: Methods for predicting prognosis in breast cancer patients using c-Met enriched CTC. Applicant: 에이비온 주식회사. The sequence listing filed with the application follows.

SEQUENCE LISTING (12 sequences)

SEQ ID NO: 1 - protein, 13 aa, synthetic construct
  REGION 1..13: note = VL-CDR1 of anti c-Met antibody A8
TGSSSNIGNNNVY

SEQ ID NO: 2 - protein, 7 aa, synthetic construct
  REGION 1..7: note = VL-CDR2 of anti c-Met antibody A8
ANSHRPS

SEQ ID NO: 3 - protein, 9 aa, synthetic construct
  REGION 1..9: note = VL-CDR3 of anti c-Met antibody A8
GSWDYSLNG

SEQ ID NO: 4 - protein, 5 aa, synthetic construct
  REGION 1..5: note = VH-CDR1 of anti c-Met antibody A8
DYYMS

SEQ ID NO: 5 - protein, 16 aa, synthetic construct
  REGION 1..16: note = VH-CDR2 of anti c-Met antibody A8
AISHDDSSIYYADSVK

SEQ ID NO: 6 - protein, 18 aa, synthetic construct
  REGION 1..18: note = VH-CDR3 of anti c-Met antibody A8
DLLQCNSEQCYSDNGMDV

SEQ ID NO: 7 - protein, 13 aa, synthetic construct
  REGION 1..13: note = VL-CDR1 of anti c-Met antibody A11
SGSSSNIGSNYVY

SEQ ID NO: 8 - protein, 7 aa, synthetic construct
  REGION 1..7: note = VL-CDR2 of anti c-Met antibody A11
ANSHRPS

SEQ ID NO: 9 - protein, 9 aa, synthetic construct
  REGION 1..9: note = VL-CDR3 of anti c-Met antibody A11
GTWDSSLNG

SEQ ID NO: 10 - protein, 5 aa, synthetic construct
  REGION 1..5: note = VH-CDR1 of anti c-Met antibody A11
DYAMS

SEQ ID NO: 11 - protein, 16 aa, synthetic construct
  REGION 1..16: note = VH-CDR2 of anti c-Met antibody A11
GISPDDSSTYYADSVK

SEQ ID NO: 12 - protein, 12 aa, synthetic construct
  REGION 1..12: note = VH-CDR3 of anti c-Met antibody A11
DVYLTETNAFDY